European Patent Application EP 4 537 833 A1, published April 16, 2025. Title: PHARMACEUTICAL COMPOSITION FOR FIBROSIS TREATMENT. Applicant: KYORIN PHARMACEUTICAL CO., LTD. Application WO PCT/JP2022/044980, filed December 6, 2022. The sequence listing filed with the application follows.

SEQUENCE LISTING (36 sequences)

SEQ ID NO: 1 - DNA, 4957 bp, Homo sapiens
  source 1..4957: mol_type = genomic DNA
gcggtccgtgcggaggctgagccggccgcgggcgcgaccggaggcagtttccgttactatggcaatgacggcagggactacaacaacctttcctatgagcaaccatacccgggaaagagtgactgtagccaagctcacattggagaatttttatagcaacctaattttacagcatgaagagagagaaaccaggcagaagaaattagaagtggccatggaagaagaaggattagcagatgaagagaaaaagttacgtcgatcacaacacgctcgcaaagaaacagagttcttacggctcaaaaggaccagacttggcttggatgactttgagtctctgaaagttataggaagaggagcttttggagaggtgcggttggtccagaagaaagatacaggccatatctatgcaatgaagatattgagaaagtctgatatgcttgaaaaagagcaggtggcccatatccgagcagaaagagatattttggtagaagcagatggtgcctgggtggtgaagatgttttacagttttcaggataagaggaatctttatctaatcatggaatttctccctggaggtgacatgatgacattgctaatgaagaaagacaccttgacagaagaggaaacacagttctacatttcagagactgttctggcaatagatgcgatccaccagttgggtttcatccatcgggatattaagccagacaaccttttattggatgccaagggtcatgtaaaattatctgattttggtttatgtacgggattaaagaaagctcacaggactgaattttatagaaatctcacacacaacccaccaagtgacttctcatttcagaacatgaactcaaagaggaaagcagaaacttggaagaagaacaggagacaactggcatattccacagttgggacaccagattacattgctccagaagtattcatgcagactggttacaacaaattgtgtgactggtggtctttgggagtgattatgtatgaaatgctaataggatatccacctttctgctctgaaacacctcaagaaacgtacagaaaagtgatgaactggaaagaaactctggtatttcctccagaggtacctatatctgagaaagccaaggacttaattctcagattttgtattgattctgaaaacagaattggaaatagtggagtagaagaaataaaaggtcatcccttttttgaaggtgtcgactgggagcacataagggaaaggccagcagcaatccctatagaaatcaaaagcattgatgatacttcaaattttgatgacttccctgaatctgatattttacaaccagtgccaaataccacagaaccggactacaaatccaaagactgggtttttctcaattatacctataaaaggtttgaagggttgactcaacgtggctctatccccacctacatgaaagctgggaagttatgaatgaagataacattcacccataaccaagagaactcaggtagctgcatcaccaggcttgcttggcgtagataacaatacactgaaatactcctgaagatggtggtgcttattgactacaagaggaaattctacaggattaggatttctaagactactataggaattggttggcagtgccagctggctcttttttttaatattttattatttttgttaactttattatatgaaggtactggaataaaaggaacagacatccctttctaactgcactgcctacatgcgtattaaggtccattctgcctgtgtgtgctgtggctttgaactgtaacacctctaatcaattcaggagaaacacatatcatttaaagcaacataggctaacctgtaggtaacactgcagtattgatgttttactgcaaatcttatgggtctagataatcagtaaaagccatcttccatagttggtgttagaacattgccctattggtttggacatctgtagaatatatatgaagacaatttctgtaatggttttaagagatttaaaaagaaattcactggttctttacaaaatagaatttatcatcaagttattacacaaacttcacagtaaggagtgacaagtttataataaggaagacaaagtttaacaccttcactcaagcactccactaatatatttacgttgcattcagaaatactgatgaccttcatatacgtagtctgtatactcatagggagatgtactgtattatataacatgtaaagttgattttcttgtgacaagagaacttctttttttaacaagaggacatggcattattttaatttgattatggtgagttgaatttaagacatgaccatgaaggctgcttgtagaattagtgtatttttattaaactatttttttaaatgtcaaacttctatcatgtaaatggacttatagagaacaaaaagctatttactttggttttctagaaagttgttacatatcatggctggttaacttttatttcttttgatgaaaatttttcctttgatagtacttgtattattgtgccattattttcttatgctccaaatgtaccaaagatcttgaacagagtggatgttcacaactgagtagaattttcctttcctgtgggcatgctgtattcagacctgacagatctttgatagaggtcagcttattaaagggcaatattgttcttgtttagctacatcactgtggtgaatatagatggaattaaggaagtaaatgcaggccagggggttgtgatgagaggataggggagataatatcagcatcaaattctttgggtatctctctaagaattaaataatcttttctagcttaatattttaattctaattcaaacaactctgaggttttggtttcattagtaatagttgaggaataatatactagcaaagaatggcctaatgtttgtcataactgttaatggatgaaattttttaaagatacaaccatgataaccattataaatgatctatgatcaaaatctaaagtgatgaattatttgtaggaatgtcttcctaatggggaagaattgcataggagcattatgcaaatctacacaagcttttataaatgttgctgctgggtagctccacagtgtttcataaggccatcctgtttcccccaactcccccatttttggtttgtttctttttaaatatttgttgagtacttacgtgtttatctaacagttcacttccatttttctagtctggattttttgagtatttaggaaagagagctattaaaaactggggatttctcaatgtgactaactctaatttttctaattataactgcctttaattaacataatattaacttttgctgaggtttatgagattttctcaccccacatcgctcccctttttttaaaaaggactgttttgctagtgtgataatgaataggtaagatatgagataattgcaacattgtctagttctagtatggtaactattcttgaaatggtattgaaaaataccgttaattcaaattgacagagattgataaaaagaaactgatttacctaagtttactttttaattgcataatagagcattttttgttttgagttccctcattcttattaccagaaagagcttgcaaatagttttactttcttggcactggaagggtagttctggaaagctactttgttgagagtctcattcttccctggagttaatagagtgattcacaatctttggggttttctcctcatcaaaagcatttcttaagtgcctatctaaaagcaattaaagactgtgtctgccctttagaagctaagaatttgattcatgatgcaaattaactagataatttgcaaagtacccttgagattgaattttctctattatatatttcccatatttcaggtgaataatttaatttaaatgacaaaaccctatctagtcaactgggcataatgacattttctttaaattagactctattttgaattaaaagagttttattataaaccgtgtgtttttggtttttctaagtatatagaaagcttgtataattcagatttatcaatttcctgatttaatgtagactttgacttttttattaaaaacctttgtattaaagcaagttatgttatttttcttttatgcatttattactaacatagctttaaatctttaaatgtattgaagcattgtgctgtctgaaaataaggaattgcttataaaccagccacttctgaatacaatatgtagctgatttaataagctagttagtgaatggaaaataagtgtggagtattaaaaatgttctttggttggtaaggcctaagatagggtttcatttatttctatactttttctgttttttaaacacctgcatatttttatgtaaatctctaaatttaaaatattttaagtacatttatttttggtgttttattgtataaaaccttagacaatcaatcagtcagtctttactgacaggagcagcagctatctgtcttttgctgatctacaaataaatgaattgagaatttagtccatagaggtccctggctaccaaacacattctcctttgaattgttaaaattcagaacattcaaaataactgttttgctacaacccatgattattttcctgttgtgtttatttaaatttactttctctttagaagtgcacttatttctgaaaaatcttaatgaaacaaacgcttagaacaaatataaatatgagacacttgggactactagagatattttagatttttatgaaaaaaatgtgaggggatattgctgctttaaaaaggaataaagtaataaaaatatatctcagctatttttttaaagcaatataattcagcaattgtctagaaaagtaatcatgaggctactgagtttggtgttcagttactgagtttcaaaaatgttttggtggcatgaggacaaaatttcattgaaggtaagataagaataaaaactatgtttacaaaa

SEQ ID NO: 2 - DNA, 4617 bp, Mus musculus
  source 1..4617: mol_type = genomic DNA
gcggccgctttggcaccgcctcacggggcgggacgaggcggggcctggcgcgagagacgcgcgccgcgggctgcggtgactgaggaggaggctgagcgggcgcgggcgacaccggcagttccagttactatggcaatgacggcaggggcaacaactacctttcctatgagcaaccatacccgggaaagagtaactgtggccaagctcacactggagaatttttacagcaacctaattttacagcatgaagagagagaaaccaggcagaagaagttagaagtggctatggaagaagaaggattggcagatgaggagaaaaagttacgtcgatcgcagcatgctcgtaaagaaacagagttcttacgccttaagaggaccagacttggcctagatgactttgagtctctgaaggttataggaagaggagctttcggagaggtgcggctggtccagaagaaagacacggggcacatctatgccatgaagatcctgaggaaagctgacatgcttgagaaagagcaggtggctcatatccgagcagaaagggacattttggtggaagcagatggagcctgggtggtgaagatgttctacagttttcaggacaaacggaatctctatctcatcatggaatttcttcctggaggtgacatgatgacattgctgatgaagaaggacaccttaacagaagaagagacacagttctacatctcagagactgtcttggcgatagatgcaattcaccagctgggcttcatccaccgggacgtcaaaccagacaaccttttactggatgccaagggacatgtaaaattatctgattttggtttgtgcacggggttaaagaaagctcacaggactgaattctacagaaacctcacacataacccgccaagcgacttctcatttcagaacatgaattcaaagcggaaagcagagacatggaagaagaacaggagacagctggcttactccacagttggaacaccagactacattgctccagaagtattcatgcagactggctacaacaaattgtgtgactggtggtccttgggagtgattatgtacgagatgctaataggctttccacctttctgctctgaaacaccacaagaaacatacagaaaagttatgagctggaaggagactctggcatttcctccggaagtgcccgtctctgagaaagccaaggacttgattctcagattttgtactgattctgaaaacagaattgggaatggtggtgtggaagaaatcaaaggtcatccgttctttgagggtgtagactgggggcacataagggaaagaccagcagctattcctatagaaatccggagtatagatgacacctcaaactttgatgacttccctgagtctgatatcttacagccagtgccgaataccacagagcccgactacaaatccaaagactgggtttttctcaattacacctacaaaaggtttgaagggctgacccagagaggctccattcctacatacatgaaagctgggaagttatgatgatcacagtcgcccatagccaggagaactcaggtagctgcatccgcaggctggctcggcatcagcaccaggagctctgggacagtgctgctctccagccagaggaacgactacagcttgggaatctgaggctgctatggctatgggaattgctcagcttttttttttctttttctttttttttgtattaactttattatacaaaggtactggaacaaaagaaacagacattccctcctaactgcactgcctacgtgcatgttgagaggtccatcctgcccatgtgctgcgcttccgattgcaacactaatccagccagaactgcattgcactgacggcaccatgacagcctgaggttgctctcagtgtccctgcttcactgcagagcccgtgggtctagaatcagtgaaaagccatcttctgtagctgctgttagtagaacatttgccctgttggtttggacattgtgggctctacatgaagacagtttctgtaccggctccaaggaacttaaggacgctgacttcaacgacattagaatttcctgtcaggctctcacgcagaccctgtgatagggaagatgagcttctgttagggtgagggcatttctcaccttcgctccggcatctccaaggctgacggtgctgagagattgtgacttgacgactgatgtgcacacatggagatggacctgaatgattgtcagctactcacttttaacaatgctgtagcattgttttagtttgaggatggtgagctgagtttcagaaatgaccatgaaagctgcttgtagaacctagtatgtttttattaaactattttttttaatgtcaaacttctgatcagtcaatggacactgtggagagcagagtgtggctcactgtggctttctgcagaggtggtacttgtccagctggtgaccctttgttcccttgattgcactagtgccattgttttccaatgaaccaaagatcctgaacagtggctgtcagcagggagtggagctccggctttacaggggagctgcgctcccttgacagaggccagccctgttcactgttagctcatcactgtggttaaagcccattatgaaatacaggaagtgggtgctggctgggagggtgtgactggagactgggcagaaaagtcagcatcagattcttggggtgtttccctaaggattacatcatcttttcttgcttagcattttgattctgaaacaactttctgaggagatgtagttttgtgagttgtagttgtagtaacttctcagggaatggctaatgtttatcatctatgattgatatagtgagactttatgggaggaatgcttctcctgagggcactgagcaatgccttgtgacccctctttcatcaaggccatcagctcctgatttattttggtgagtcctttaaggccccccccattttgctgttgagtctggtaatcaacaccacttgttatctactggctcagctgtagcctgatcaatcctatgccaagtatttggagaaagcactgaaaatggtagataagcctccctgactttagctgccttaatatctgcagggtatatgagcttctccaagtagtctgtctcaagggtacttaagcagcagagacccctgaatatagggattctaccttttcttttagaatgggacttttctagtgtgagtgtctaggttggataggagaccttgccaaattctctagctcaggtgtgataactacctaactatcgtagggtgggtgttgtcaatccaggtaactggggtagtttgagattagtgtacaggagaattaccaaacttatgtttccatgatgtagggacagagcactttgtctgatctctctgttgtggttgtaaaagctgtgagaggcaggtttcctggtggtggagaggcattttgggaagtttgctttgcagcattaacatggctgcccacttttcaggaatttcttgtggaagcgttccctaagctagtgtaaggcccctaaagactgtctgcctgttgaagcaaaaatacgaggcatggtgcaaattgtgcaaataatttgcagagatcctctgatactgactttttcccattatacacttcccatattttaggtaaataatgtaatttaagtgataaaaccctatcttaatcaactgggcatagtgacattttctcttaatctctattttgagtctaggaagttttattataaacggtggtttgggtttttctaaagatacagaaaatgtgtataatccagatgtattggtttcctgattgagtagagacttgtactttttcattaaaacctttgtgttgaagcagttgttcacagctaagtctggagatgtatgaaacctgggctgtccaaagtaagttgtgaccacttaaccaccgatcagctgtgtggtgaaagtgccagctatggaatattaaatgcgttctttggctgctaaggcttaagatagggctcctttatttccgtatcagcatagctcttaaacacatgcatagctctgtacaagctgtacattttaaaatatcttgaagcacagtttgttttggtgttgagaatctagtccaccagtcagtctctgacagcaggagagatagctagccacctacctatcttttggcagtctacaagtaagttacttgagggtcagaaaagggtcctggcacatcctctctttgaattgttaaaatttggaaaattcaaaagcaactgttttgctatgatcatgattatttctcattttatttcaaaattattttctctgtagaagtgcacttatttctgaaaaatcttaagccaacacttaataaatatgagacacttgagactactagaaatattttagatttttattacaaaatgtgaggagatgaaggaataaagtaatagaagtgtattgtagtttttgggggggttttgtttgtttttttttttaagcaatataatccagcagttgtccagaaccatcaggcttctgagcccatccagcgtttcgaagactgttgggcaggggcattgagggcctcttcattcacggcacaacgagaataaagccacgtttacaaagctctgt

SEQ ID NO: 3 - DNA, 16 bp, synthetic construct
  source 1..16: mol_type = other DNA
cagttgactagatagg

SEQ ID NO: 4 - DNA, 16 bp, synthetic construct
  source 1..16: mol_type = other DNA
gatcgacgtaactttt

SEQ ID NO: 5 - DNA, 16 bp, synthetic construct
  source 1..16: mol_type = other DNA
ttaaccagccatgata

SEQ ID NO: 6 - DNA, 16 bp, synthetic construct
  source 1..16: mol_type = other DNA
ccatcttcaggagtat

SEQ ID NO: 7 - DNA, 16 bp, synthetic construct
  source 1..16: mol_type = other DNA
attagtggagtgcttg

SEQ ID NO: 8 - DNA, 16 bp, synthetic construct
  source 1..16: mol_type = other DNA
tgtgatcgacgtaact

SEQ ID NO: 9 - DNA, 16 bp, synthetic construct
  source 1..16: mol_type = other DNA
gtggagtgcttgagtg

SEQ ID NO: 10 - DNA, 16 bp, synthetic construct
  source 1..16: mol_type = other DNA
gtaataacttgatgat

SEQ ID NO: 11 - DNA, 16 bp, synthetic construct
  source 1..16: mol_type = other DNA
gaattgattagaggtg

SEQ ID NO: 12 - DNA, 16 bp, synthetic construct
  source 1..16: mol_type = other DNA
gacaattgctgaatta

SEQ ID NO: 13 - DNA, 16 bp, synthetic construct
  source 1..16: mol_type = other DNA
taggcagtgcagttag

SEQ ID NO: 14 - DNA, 16 bp, synthetic construct
  source 1..16: mol_type = other DNA
tatgcccagttgatta

SEQ ID NO: 15 - DNA, 16 bp, synthetic construct
  source 1..16: mol_type = other DNA
agttgattaagatagg

SEQ ID NO: 16 - DNA, 16 bp, synthetic construct
  source 1..16: mol_type = other DNA
gacaactgctggatta

SEQ ID NO: 17 - DNA, 16 bp, synthetic construct
  source 1..16: mol_type = other DNA
ttacctggattgacaa

SEQ ID NO: 18 - DNA, 16 bp, synthetic construct
  source 1..16: mol_type = other DNA
actagtgcaatcaagg

SEQ ID NO: 19 - DNA, 16 bp, synthetic construct
  source 1..16: mol_type = other DNA
catcagtcgtcaagtc

SEQ ID NO: 20 - DNA, 16 bp, synthetic construct
  source 1..16: mol_type = other DNA
tcacacctgagctaga

SEQ ID NO: 21 - DNA, 16 bp, synthetic construct
  source 1..16: mol_type = other DNA
agatagagattccgtt

SEQ ID NO: 22 - DNA, 16 bp, synthetic construct
  source 1..16: mol_type = other DNA
cactggctgtaagata

SEQ ID NO: 23 - RNA, 19 nt, synthetic construct
  source 1..19: mol_type = other RNA
ttctttgcgagcgtgttgt

SEQ ID NO: 24 - RNA, 19 nt, synthetic construct
  source 1..19: mol_type = other RNA
aaataccagagtttctttc

SEQ ID NO: 25 - RNA, 19 nt, synthetic construct
  source 1..19: mol_type = other RNA
aaatgtagaactgtgtttc

SEQ ID NO: 26 - RNA, 19 nt, synthetic construct
  source 1..19: mol_type = other RNA
tttgttgtaaccagtctgc

SEQ ID NO: 27 - DNA, 21 bp, synthetic construct
  source 1..21: mol_type = other DNA
  misc_feature 1..19: note = RNA
tgagtcaacccttcaaacctt

SEQ ID NO: 28 - DNA, 21 bp, synthetic construct
  source 1..21: mol_type = other DNA
  misc_feature 1..19: note = RNA
tccagtaaaaggttgtctggt

SEQ ID NO: 29 - DNA, 21 bp, synthetic construct
  source 1..21: mol_type = other DNA
  misc_feature 1..19: note = RNA
tactctttcccgggtatggtt

SEQ ID NO: 30 - RNA, 19 nt, synthetic construct
  source 1..19: mol_type = other RNA
acaacacgctcgcaaagaa

SEQ ID NO: 31 - RNA, 19 nt, synthetic construct
  source 1..19: mol_type = other RNA
gaaagaaactctggtattt

SEQ ID NO: 32 - RNA, 19 nt, synthetic construct
  source 1..19: mol_type = other RNA
gaaacacagttctacattt

SEQ ID NO: 33 - RNA, 19 nt, synthetic construct
  source 1..19: mol_type = other RNA
gcagactggttacaacaaa

SEQ ID NO: 34 - DNA, 21 bp, synthetic construct
  source 1..21: mol_type = other DNA
  misc_feature 1..19: note = RNA
ggtttgaagggttgactcatt

SEQ ID NO: 35 - DNA, 21 bp, synthetic construct
  source 1..21: mol_type = other DNA
  misc_feature 1..19: note = RNA
cagacaaccttttactggatt

SEQ ID NO: 36 - DNA, 21 bp, synthetic construct
  source 1..21: mol_type = other DNA
  misc_feature 1..19: note = RNA
ccatacccgggaaagagtatt